European Patent Application EP 4 276 177 A1, published November 15, 2023. Title: Novel citrate synthase variant and a method for producing O-Acetyl-L-Homoserine or L-Methionine using the same. Applicant: CJ CheilJedang Corporation. The sequence listing filed with the application follows.

SEQUENCE LISTING (33 sequences)

SEQ ID NO: 1 - protein, 437 aa, Unknown [sequence omitted]

SEQ ID NO: 2 - DNA, 1314 bp, Unknown
  ATCC13032 GltA NT
atgtttgaaagggatatcgtggctactgataacaacaaggctgtcctgcactaccccggtggcgagttcgaaatggacatcatcgaggcttctgagggtaacaacggtgttgtcctgggcaagatgctgtctgagactggactgatcacttttgacccaggttatgtgagcactggctccaccgagtcgaagatcacctacatcgatggcgatgcgggaatcctgcgttaccgcggctatgacatcgctgatctggctgagaatgccaccttcaacgaggtttcttacctacttatcaacggtgagctaccaaccccagatgagcttcacaagtttaacgacgagattcgccaccacacccttctggacgaggacttcaagtcccagttcaacgtgttcccacgcgacgctcacccaatggcaaccttggcttcctcggttaacattttgtctacctactaccaggaccagctgaacccactcgatgaggcacagcttgataaggcaaccgttcgcctcatggcaaaggttccaatgctggctgcgtacgcacaccgcgcacgcaagggtgctccttacatgtacccagacaactccctcaatgcgcgtgagaacttcctgcgcatgatgttcggttacccaaccgagccatacgagatcgacccaatcatggtcaaggctctggacaagctgctcatcctgcacgctgaccacgagcagaactgctccacctccaccgttcgtatgatcggttccgcacaggccaacatgtttgtctccatcgctggtggcatcaacgctctgtccggcccactgcacggtggcgcaaaccaggctgttctggagatgctcgaagacatcaagagcaaccacggtggcgacgcaaccgagttcatgaacaaggtcaagaacaaggaagacggcgtccgcctcatgggcttcggacaccgcgtttacaagaactacgatccacgtgcagcaatcgtcaaggagaccgcacacgagatcctcgagcacctcggtggcgacgatcttctggatctggcaatcaagctggaagaaattgcactggctgatgattacttcatctcccgcaagctctacccgaacgtagacttctacaccggcctgatctaccgcgcaatgggcttcccaactgacttcttcaccgtattgttcgcaatcggtcgtctgccaggatggatcgctcactaccgcgagcagctcggtgcagcaggcaacaagatcaaccgcccacgccaggtctacaccggcaacgaatcccgcaagttggttcctcgcgaggagcgctaa

SEQ ID NO: 3 - protein, 54 aa, Unknown
  ATCC 13032 GltA K415H 362~415
FISRKLYPNVDFYTGLIYRAMGFPTDFFTVLFAIGRLPGWIAHYREQLGAAGNH

SEQ ID NO: 4 - protein, 437 aa, Artificial Sequence
  ATCC13032 GltA K415H AA
MFERDIVATDNNKAVLHYPGGEFEMDIIEASEGNNGVVLGKMLSETGLITFDPGYVSTGSTESKITYIDGDAGILRYRGYDIADLAENATFNEVSYLLINGELPTPDELHKFNDEIRHHTLLDEDFKSQFNVFPRDAHPMATLASSVNILSTYYQDQLNPLDEAQLDKATVRLMAKVPMLAAYAHRARKGAPYMYPDNSLNARENFLRMMFGYPTEPYEIDPIMVKALDKLLILHADHEQNCSTSTVRMIGSAQANMFVSIAGGINALSGPLHGGANQAVLEMLEDIKSNHGGDATEFMNKVKNKEDGVRLMGFGHRVYKNYDPRAAIVKETAHEILEHLGGDDLLDLAIKLEEIALADDYFISRKLYPNVDFYTGLIYRAMGFPTDFFTVLFAIGRLPGWIAHYREQLGAAGNHINRPRQVYTGNESRKLVPREER

SEQ ID NO: 5 - DNA, 1314 bp, Artificial Sequence
  ATCC13032 GltA K415H NT
atgtttgaaagggatatcgtggctactgataacaacaaggctgtcctgcactaccccggtggcgagttcgaaatggacatcatcgaggcttctgagggtaacaacggtgttgtcctgggcaagatgctgtctgagactggactgatcacttttgacccaggttatgtgagcactggctccaccgagtcgaagatcacctacatcgatggcgatgcgggaatcctgcgttaccgcggctatgacatcgctgatctggctgagaatgccaccttcaacgaggtttcttacctacttatcaacggtgagctaccaaccccagatgagcttcacaagtttaacgacgagattcgccaccacacccttctggacgaggacttcaagtcccagttcaacgtgttcccacgcgacgctcacccaatggcaaccttggcttcctcggttaacattttgtctacctactaccaggaccagctgaacccactcgatgaggcacagcttgataaggcaaccgttcgcctcatggcaaaggttccaatgctggctgcgtacgcacaccgcgcacgcaagggtgctccttacatgtacccagacaactccctcaatgcgcgtgagaacttcctgcgcatgatgttcggttacccaaccgagccatacgagatcgacccaatcatggtcaaggctctggacaagctgctcatcctgcacgctgaccacgagcagaactgctccacctccaccgttcgtatgatcggttccgcacaggccaacatgtttgtctccatcgctggtggcatcaacgctctgtccggcccactgcacggtggcgcaaaccaggctgttctggagatgctcgaagacatcaagagcaaccacggtggcgacgcaaccgagttcatgaacaaggtcaagaacaaggaagacggcgtccgcctcatgggcttcggacaccgcgtttacaagaactacgatccacgtgcagcaatcgtcaaggagaccgcacacgagatcctcgagcacctcggtggcgacgatcttctggatctggcaatcaagctggaagaaattgcactggctgatgattacttcatctcccgcaagctctacccgaacgtagacttctacaccggcctgatctaccgcgcaatgggcttcccaactgacttcttcaccgtattgttcgcaatcggtcgtctgccaggatggatcgctcactaccgcgagcagctcggtgcagcaggcaaccacatcaaccgcccacgccaggtctacaccggcaacgaatcccgcaagttggttcctcgcgaggagcgctaa

SEQ ID NO: 6 - protein, 437 aa, Artificial Sequence
  ATCC13032 GltA K415H+ N241T AA
MFERDIVATDNNKAVLHYPGGEFEMDIIEASEGNNGVVLGKMLSETGLITFDPGYVSTGSTESKITYIDGDAGILRYRGYDIADLAENATFNEVSYLLINGELPTPDELHKFNDEIRHHTLLDEDFKSQFNVFPRDAHPMATLASSVNILSTYYQDQLNPLDEAQLDKATVRLMAKVPMLAAYAHRARKGAPYMYPDNSLNARENFLRMMFGYPTEPYEIDPIMVKALDKLLILHADHEQTCSTSTVRMIGSAQANMFVSIAGGINALSGPLHGGANQAVLEMLEDIKSNHGGDATEFMNKVKNKEDGVRLMGFGHRVYKNYDPRAAIVKETAHEILEHLGGDDLLDLAIKLEEIALADDYFISRKLYPNVDFYTGLIYRAMGFPTDFFTVLFAIGRLPGWIAHYREQLGAAGNHINRPRQVYTGNESRKLVPREER

SEQ ID NO: 7 - DNA, 1314 bp, Artificial Sequence
  ATCC13032 GltA K415H+ N241T NT
atgtttgaaagggatatcgtggctactgataacaacaaggctgtcctgcactaccccggtggcgagttcgaaatggacatcatcgaggcttctgagggtaacaacggtgttgtcctgggcaagatgctgtctgagactggactgatcacttttgacccaggttatgtgagcactggctccaccgagtcgaagatcacctacatcgatggcgatgcgggaatcctgcgttaccgcggctatgacatcgctgatctggctgagaatgccaccttcaacgaggtttcttacctacttatcaacggtgagctaccaaccccagatgagcttcacaagtttaacgacgagattcgccaccacacccttctggacgaggacttcaagtcccagttcaacgtgttcccacgcgacgctcacccaatggcaaccttggcttcctcggttaacattttgtctacctactaccaggaccagctgaacccactcgatgaggcacagcttgataaggcaaccgttcgcctcatggcaaaggttccaatgctggctgcgtacgcacaccgcgcacgcaagggtgctccttacatgtacccagacaactccctcaatgcgcgtgagaacttcctgcgcatgatgttcggttacccaaccgagccatacgagatcgacccaatcatggtcaaggctctggacaagctgctcatcctgcacgctgaccacgagcagacctgctccacctccaccgttcgtatgatcggttccgcacaggccaacatgtttgtctccatcgctggtggcatcaacgctctgtccggcccactgcacggtggcgcaaaccaggctgttctggagatgctcgaagacatcaagagcaaccacggtggcgacgcaaccgagttcatgaacaaggtcaagaacaaggaagacggcgtccgcctcatgggcttcggacaccgcgtttacaagaactacgatccacgtgcagcaatcgtcaaggagaccgcacacgagatcctcgagcacctcggtggcgacgatcttctggatctggcaatcaagctggaagaaattgcactggctgatgattacttcatctcccgcaagctctacccgaacgtagacttctacaccggcctgatctaccgcgcaatgggcttcccaactgacttcttcaccgtattgttcgcaatcggtcgtctgccaggatggatcgctcactaccgcgagcagctcggtgcagcaggcaaccacatcaaccgcccacgccaggtctacaccggcaacgaatcccgcaagttggttcctcgcgaggagcgctaa

SEQ ID NO: 8 - DNA, 44 bp, Artificial Sequence
  primer 1
tcgagctcggtacccccgttcgtatgatcggttccgcacaggcc

SEQ ID NO: 9 - DNA, 31 bp, Artificial Sequence
  primer 2
gtgcagcaggcaaccacatcaaccgcccacg

SEQ ID NO: 10 - DNA, 31 bp, Artificial Sequence
  primer 3
cgtgggcggttgatgtggttgcctgctgcac

SEQ ID NO: 11 - DNA, 46 bp, Artificial Sequence
  primer 4
ctctagaggatccccgccgtaagcagcctctggtggaatggtcagc

SEQ ID NO: 12 - DNA, 35 bp, Artificial Sequence
  primer 5
gctgaccacgagcagacctgctccacctccaccgt

SEQ ID NO: 13 - DNA, 35 bp, Artificial Sequence
  primer 6
acggtggaggtggagcaggtctgctcgtggtcagc

SEQ ID NO: 14 - protein, 418 aa, Unknown
  YjeH AA
MSGLKQELGLAQGIGLLSTSLLGTGVFAVPALAALVAGNNSLWAWPVLIILVFPIAIVFAILGRHYPSAGGVAHFVGMAFGSRLERVTGWLFLSVIPVGLPAALQIAAGFGQAMFGWHSWQLLLAELGTLALVWYIGTRGASSSANLQTVIAGLIVALIVAIWWAGDIKPANIPFPAPGNIELTGLFAALSVMFWCFVGLEAFAHLASEFKNPERDFPRALMIGLLLAGLVYWGCTVVVLHFDAYGEKMAAAASLPKIVVQLFGVGALWIACVIGYLACFASLNIYIQSFARLVWSQAQHNPDHYLARLSSRHIPNNALNAVLGCCVVSTLVIHALEINLDALIIYANGIFIMIYLLCMLAGCKLLQGRYRLLAVVGGLLCVLLLAMVGWKSLYALIMLAGLWLLLPKRKTPENGITT

SEQ ID NO: 15 - DNA, 1257 bp, Unknown
  YjeH NT
atgagtggactcaaacaagaactggggctggcccagggcattggcctgctatcgacgtcattattaggcactggcgtgtttgccgttcctgcgttagctgcgctggtagcgggcaataacagcctgtgggcgtggcccgttttgattatcttagtgttcccgattgcgattgtgtttgcgattctgggtcgccactatcccagcgcaggcggcgtcgcgcacttcgtcggtatggcgtttggttcgcggcttgagcgagtcaccggctggctgtttttatcggtcattcccgtgggtttgcctgccgcactacaaattgccgccgggttcggccaggcgatgtttggctggcatagctggcaactgttgttggcagaactcggtacgctggcgctggtgtggtatatcggtactcgcggtgccagttccagtgctaatctacaaaccgttattgccggacttatcgtcgcgctgattgtcgctatctggtgggcgggcgatatcaaacctgcgaatatcccctttccggcacctggtaatatcgaacttaccgggttatttgctgcgttatcagtgatgttctggtgttttgtcggtctggaggcatttgcccatctcgcctcggaatttaaaaatccagagcgtgattttcctcgtgctttgatgattggtctgctgctggcaggattagtctactggggctgtacggtagtcgtcttacacttcgacgcctatggtgaaaaaatggcggcggcagcatcgcttccaaaaattgtagtgcagttgttcggtgtaggagcgttatggattgcctgcgtgattggctatctggcctgctttgccagtctcaacatttatatacagagcttcgcccgcctggtctggtcgcaggcgcaacataatcctgaccactacctggcacgcctctcttctcgccatatcccgaataatgccctcaatgcggtgctcggctgctgtgtggtgagcactttggtgattcatgctttagagatcaatctggacgctcttattatttatgccaatggcatctttattatgatttatctgttatgcatgctggcaggctgtaaattattgcaaggacgttatcgactactggcggtggttggcgggctgttatgcgttctgttactggcaatggtcggctggaaaagtctctatgcgctgatcatgctggcggggttatggctgttgctgccaaaacgaaaaacgccggaaaatggcataaccacataa

SEQ ID NO: 16 - protein, 88 aa, Unknown
  NCgl2335 AA
MAYTFDHVVAWRWCTKEDAYNYTHLFDQLQPPLIVTTDGQKRRTQSHHHDLADNENPTLPRPRQTQRPKTRHPKTRAELAEKHSGVSP

SEQ ID NO: 17 - DNA, 267 bp, Unknown
  NCgl2335 NT
gtggcctacaccttcgaccacgtcgtcgcctggcgctggtgcaccaaagaagacgcctacaactacacccacctcttcgatcaactccaaccacccttaatcgtgaccaccgacggacaaaaaaggcgcactcaaagccatcaccacgacctggccgacaacgaaaatccaacgctgcctcgtccacgtcaaacgcaacgtccaaaaacacgtcaccctaagacccgtgctgagctcgccgaaaagcactccggggtctctccttga

SEQ ID NO: 18 - DNA, 39 bp, Artificial Sequence
  Tn_5 F
tgaattcgagctcggtaccccaccgacgcgcatctgcct

SEQ ID NO: 19 - DNA, 50 bp, Artificial Sequence
  Tn_5 R
ggtgtggtgactttcagcagttcccgggggggaggaggcatgtggtgttg

SEQ ID NO: 20 - DNA, 50 bp, Artificial Sequence
  Tn_3 F
caacaccacatgcctcctcccccccgggaactgctgaaagtcaccacacc

SEQ ID NO: 21 - DNA, 42 bp, Artificial Sequence
  Tn_3 R
gtcgactctagaggatccccctcccaaaccattgaggaatgg

SEQ ID NO: 22 - DNA, 39 bp, Artificial Sequence
  CJ7_yjeH F
acaccacatgcctcctccccagaaacatcccagcgctac

SEQ ID NO: 23 - DNA, 43 bp, Artificial Sequence
  CJ7_yjeH R
agttcttgtttgagtccactcatagtgtttcctttcgttgggt

SEQ ID NO: 24 - DNA, 44 bp, Artificial Sequence
  yjeH F
acccaacgaaaggaaacactatgagtggactcaaacaagaactg

SEQ ID NO: 25 - DNA, 44 bp, Artificial Sequence
  yjeH R
gactttcagcagttcccgggttatgtggttatgccattttccgg

SEQ ID NO: 26 - protein, 418 aa, Artificial Sequence
  yjeH F351L AA
MSGLKQELGLAQGIGLLSTSLLGTGVFAVPALAALVAGNNSLWAWPVLIILVFPIAIVFAILGRHYPSAGGVAHFVGMAFGSRLERVTGWLFLSVIPVGLPAALQIAAGFGQAMFGWHSWQLLLAELGTLALVWYIGTRGASSSANLQTVIAGLIVALIVAIWWAGDIKPANIPFPAPGNIELTGLFAALSVMFWCFVGLEAFAHLASEFKNPERDFPRALMIGLLLAGLVYWGCTVVVLHFDAYGEKMAAAASLPKIVVQLFGVGALWIACVIGYLACFASLNIYIQSFARLVWSQAQHNPDHYLARLSSRHIPNNALNAVLGCCVVSTLVIHALEINLDALIIYANGILIMIYLLCMLAGCKLLQGRYRLLAVVGGLLCVLLLAMVGWKSLYALIMLAGLWLLLPKRKTPENGITT

SEQ ID NO: 27 - DNA, 1257 bp, Artificial Sequence
  yjeH F351L NT
atgagtggactcaaacaagaactggggctggcccagggcattggcctgctatcgacgtcattattaggcactggcgtgtttgccgttcctgcgttagctgcgctggtagcgggcaataacagcctgtgggcgtggcccgttttgattatcttagtgttcccgattgcgattgtgtttgcgattctgggtcgccactatcccagcgcaggcggcgtcgcgcacttcgtcggtatggcgtttggttcgcggcttgagcgagtcaccggctggctgaatttatcggtcattcccgtgggtttgcctgccgcactacaaattgccgccgggttcggccaggcgatgtttggctggcatagctggcaactgttgttggcagaactcggtacgctggcgctggtgtggtatatcggtactcgcggtgccagttccagtgctaatctacaaaccgttattgccggacttatcgtcgcgctgattgtcgctatctggtgggcgggcgatatcaaacctgcgaatatcccctttccggcacctggtaatatcgaacttaccgggttatttgctgcgttatcagtgatgttctggtgttttgtcggtctggaggcatttgcccatctcgcctcggaatttaaaaatccagagcgtgattttcctcgtgctttgatgattggtctgctgctggcaggattagtctactggggctgtacggtagtcgtcttacacttcgacgcctatggtgaaaaaatggcggcggcagcatcgcttccaaaaattgtagtgcagttgttcggtgtaggagcgttatggattgcctgcgtgattggctatctggcctgctttgccagtctcaacatttatatacagagcttcgcccgcctggtctggtcgcaggcgcaacataatcctgaccactacctggcacgcctctcttctcgccatatcccgaataatgccctcaatgcggtgctcggctgctgtgtggtgagcactttggtgattcatgctttagagatcaatctggacgctcttattatttatgccaatggcatccttattatgatttatctgttatgcatgctggcaggctgtaaattattgcaaggacgttatcgactactggcggtggttggcgggctgttatgcgttctgttactggcaatggtcggctggaaaagtctctatgcgctgatcatgctggcggggttatggctgttgctgccaaaacgaaaaacgccggaaaatggcataaccacataa

SEQ ID NO: 28 - DNA, 23 bp, Artificial Sequence
  F351L F
caatggcatccttattatgattt

SEQ ID NO: 29 - DNA, 23 bp, Artificial Sequence
  F351L R
aaatcataataaggatgccattg

SEQ ID NO: 30 - DNA, 20 bp, Artificial Sequence
  gltA-F
atgtttgaaagggatatcgt

SEQ ID NO: 31 - DNA, 21 bp, Artificial Sequence
  gltA-R
ttagcgctcctcgcgaggaac

SEQ ID NO: 32 - DNA, 5803 bp, Artificial Sequence
  pDCM2
gttcgcttgctgtccataaaaccgcccagtctagctatcgccatgtaagcccactgcaagctacctgctttctctttgcgcttgcgttttcccttgtccagatagcccagtagctgacattcatccggggtcagcaccgtttctgcggactggctttctacgtgttccgcttcctttagcagcccttgcgccctgagtgcttgcggcagcgtgaagctagcttttatcgccattcgccattcaggctgcgcaactgttgggaagggcgatcggtgcgggcctcttcgctattacgccagctggcgaaagggggatgtgctgcaaggcgattaagttgggtaacgccagggttttcccagtcacgacgttgtaaaacgacggccagtgaattcgagctcggtacccggggatcctctagagtcgacctgcaggcatgcaagcttggcgtaatcatggtcatagctgtttcctgtgtgaaattgttatccgctcacaattccacacaacatacgagccggaagcataaagtgtaaagcctggggtgcctaatgagtgagctaactcacattaattgcgttgcgctcactgcccgctttccagtcgggaaacctgtcgtgccagctgcattaatgaatcggccaacgcgcggggagaggcggtttgcgtattgggcgctcttccgcttcctcgctcactgactcgctgcgctcggtcgttcggctgcggcgagcggtatcagctcactcaaaggcggtaatacggttatccacagaatcaggggataacgcaggaaagaacatgtgagcaaaaggccagcaaaaggccaggaaccgtaaaaaggccgcgttgctggcgtttttccataggctccgcccccctgacgagcatcacaaaaatcgacgctcaagtcagaggtggcgaaacccgacaggactataaagataccaggcgtttccccctggaagctccctcgtgcgctctcctgttccgaccctgccgcttaccggatacctgtccgcctttctcccttcgggaagcgtggcgctttctcaatgctcacgctgtaggtatctcagttcggtgtaggtcgttcgctccaagctgggctgtgtgcacgaaccccccgttcagcccgaccgctgcgccttatccggtaactatcgtcttgagtccaacccggtaagacacgacttatcgccactggcagcagccactggtaacaggattagcagagcgaggtatgtaggcggtgctacagagttcttgaagtggtggcctaactacggctacactagaaggacagtatttggtatctgcgctctgctgaagccagttaccttcggaaaaagagttggtagctcttgatccggcaaacaaaccaccgctggtagcggtggtttttttgtttgcaagcagcagattacgcgcagaaaaaaaggatctcaagaagatcctttgatcttttctacggggtctgacgctcagtggaacgaaaactcacgttaagggattttggtcatgagattatcaaaaaggatcttcacctagatccttttggggtgggcgaagaactccagcatgagatccccgcgctggaggatcatccagccctgatagaaacagaagccactggagcacctcaaaaacaccatcatacactaaatcagtaagttggcagcatcacccgacgcactttgcgccgaataaatacctgtgacggaagatcacttcgcagaataaataaatcctggtgtccctgttgataccgggaagccctgggccaacttttggcgaaaatgagacgttgatcggcacgtaagaggttccaactttcaccataatgaaataagatcactaccgggcgtattttttgagttatcgagattttcaggagctgatagaaacagaagccactggagcacctcaaaaacaccatcatacactaaatcagtaagttggcagcatcacccgacgcactttgcgccgaataaatacctgtgacggaagatcacttcgcagaataaataaatcctggtgtccctgttgataccgggaagccctgggccaacttttggcgaaaatgagacgttgatcggcacgtaagaggttccaactttcaccataatgaaataagatcactaccgggcgtattttttgagttatcgagattttcaggagctctttggcatcgtctctcgcctgtcccctcagttcagtaatttcctgcatttgcctgtttccagtcggtagatattccacaaaacagcagggaagcagcgcttttccgctgcataaccctgcttcggggtcattatagcgattttttcggtatatccatcctttttcgcacgatatacaggattttgccaaagggttcgtgtagactttccttggtgtatccaacggcgtcagccgggcaggataggtgaagtaggcccacccgcgagcgggtgttccttcttcactgtcccttattcgcacctggcggtgctcaacgggaatcctgctctgcgaggctggccggctaccgccggcgtaacagatgagggcaagcggatggctgatgaaaccaagccaaccaggaagggcagcccacctatcaaggtgtactgccttccagacgaacgaagagcgattgaggaaaaggcggcggcggccggcatgagcctgtcggcctacctgctggccgtcggccagggctacaaaatcacgggcgtcgtggactatgagcacgtccgcgagggcgtcccggaaaacgattccgaagcccaacctttcatagaaggcggcggtggaatcgaaatctcgtgatggcaggttgggcgtcgcttggtcggtcatttcgaaaaaggttaggaatacggttagccatttgcctgcttttatatagttcantatgggattcacctttatgttgataagaaataaaagaaaatgccaataggatatcggcattttcttttgcgtttttatttgttaactgttaattgtccttgttcaaggatgctgtctttgacaacagatgttttcttgcctttgatgttcagcaggaagctcggcgcaaacgttgattgtttgtctgcgtagaatcctctgtttgtcatatagcttgtaatcacgacattgtttcctttcgcttgaggtacagcgaagtgtgagtaagtaaaggttacatcgttaggcggatcaagatccatttttaacacaaggccagttttgttcagcggcttgtatgggccagttaaagaattagaaacataaccaagcatgtaaatatcgttagacgtaatgccgtcaatcgtcatttttgatccgcgggagtcagtgaacaggtaccatttgccgttcattttaaagacgttcgcgcgttcaatttcatctgttactgtgttagatgcaatcagcggtttcatcacttttttcagtgtgtaatcatcgtttagctcaatcataccgagagcgccgtttgctaactcagccgtgcgttttttatcgctttgcagaagtttttgactttcttgacggaagaatgatgtgcttttgccatagtatgctttgttaaataaagattcttcgccttggtagccatcttcagttccagtgtttgcttcaaatactaagtatttgtggcctttatcttctacgtagtgaggatctctcagcgtatggttgtcgcctgagctgtagttgccttcatcgatgaactgctgtacattttgatacgtttttccgtcaccgtcaaagattgatttataatcctctacaccgttgatgttcaaagagctgtctgatgctgatacgttaacttgtgcagttgtcagtgtttgtttgccgtaatgtttaccggagaaatcagtgtagaataaacggatttttccgtcagatgtaaatgtggctgaacctgaccattcttgtgtttggtcttttaggatagaatcatttgcatcgaatttgtcgctgtctttaaagacgcggccagcgtttttccagctgtcaatagaagtttcgccgactttttgatagaacatgtaaatcgatgtgtcatccgcatttttaggatctccggctaatgcaaagacgatgtggtagccgtgatagtttgcgacagtgccgtcagcgttttgtaatggccagctgtcccaaacgtccaggccttttgcagaagagatatttttaattgtggacgaatcaaattcagaaacttgatatttttcatttttttgctgttcagggatttgcagcatatcatggcgtgtaatatgggaaatgccgtatgtttccttatatggcttttggttcgtttctttcgcaaacgcttgagttgcgcctcctgccagcagtgcggtagtaaaggttaatactgttgcttgttttgcaaactttttgatgttcatcgttcatgtctccttttttatgtactgtgttagcggtctgcttcttccagccctcctgtttgaagatggcaagttagttacgcacaataaaaaaagacctaaaatatgtaaggggtgacgccaaagtatacactttgccctttacacattttaggtcttgcctgctttatcagtaacaaacccgcgcgatttacttttcgacctcattctattagactctcgtttggattgcaactggtctattttcctcttttgtttgatagaaaatcataaaaggatttgcagactacgggcctaaagaactaaaaaatctatctgtttcttttcattctctgtattttttatagtttctgttgcatgggcataaagttgcctttttaatcacaattcagaaaatatcataatatctcatttcactaaataatagtgaacggcaggtatatgtgatgggttaaaaaggatcaccccagagtcccgctcagaagaactcgtcaagaaggcgatagaaggcgatgcgctgcgaatcgggagcggcgataccgtaaagcacgaggaagcggtcagcccattcgccgccaagctcttcagcaatatcacgggtagccaacgctatgtcctgatagcggtccgccacacccagccggccacagtcgatgaatccagaaaagcggccattttccaccatgatattcggcaagcaggcatcgccatgggtcacgacgagatcctcgccgtcgggcatccgcgccttgagcctggcgaacagttcggctggcgcgagcccctgatgctcttcgtccagatcatcctgatcgacaagaccggcttccatccgagtacgtgctcgctcgatgcgatgtttcgcttggtggtcgaatgggcaggtagccggatcaagcgtatgcagccgccgcattgcatcagccatgatggatactttctcggcaggagcaaggtgagatgacaggagatcctgccccggcacttcgcccaatagcagccagtcccttcccgcttcagtgacaacgtcgagacagctgcgcaaggaacgcccgtcgtggccagccacgatagccgcgctgcctcgtcttggagttcattcagggcaccggacaggtcggtcttgacaaaaagaaccgggcgcccctgcgctgacagccggaacacggcggcatcagagcagccgattgtctgttgtgcccagtcatagccgaatagcctctccacccaagcggccggagaacctgcgtgcaatccatcttgttcaatcatgcgaaacgatcctcatcctgtctcttgatcagatcttgatcccctgcgccatcagatccttggcggcaagaaagccatccagtttactttgcagggcttcccaaccttaccagagggcgccccagctggcaattccg

SEQ ID NO: 33 - protein, 127 aa, Artificial Sequence
  General formula 1
  MISC_FEATURE (1): Xaa is N or S.
  MISC_FEATURE (9): Xaa is A or E.
  MISC_FEATURE (73): Xaa is Y or C.
XNHGGDATXFMNKVKNKEDGVRLMGFGHRVYKNYDPRAAIVKETAHEILEHLGGDDLLDLAIKLEEIALADDXFISRKLYPNVDFYTGLIYRAMGFPTDFFTVLFAIGRLPGWIAHYREQLGAAGNH